European Patent Application EP 4 198 049 A1, published June 21, 2023. Title: BMP-9 or BMP-10 variants with improved therapeutic effect by reducing the side effects of ossicle formation and a pharmaceutical composition using the same. Applicant: NIBEC Co., Ltd. Seoul National University Industry Foundation. The sequence listing filed with the application follows.

SEQUENCE LISTING (33 sequences)

SEQ ID NO: 1 - protein, 426 aa, Artificial Sequence
  Homo sapiens
MAWVWTLLFLMAAAQSIQAKPLQSWGRGSAGGNAHSPLGVPGGGLPEHTFNLKMFLENVKVDFLRSLNLSGVPSQDKTRVEPPQYMIDLYNRYTSDKSTTPASNIVRSFSMEDAISITATEDFPFQKHILLFNISIPRHEQITRAELRLYVSCQNHVDPSHDLKGSVVIYDVLDGTDAWDSATETKTFLVSQDIQDEGWETLEVSSAVKRWVRSDSTKSKNKLEVTVESHRKGCDTLDISVPPGSRNLPFFVVFSNDHSSGTKETRLELREMISHEQESVLKKLSKDGSTEAGESSHEEDTDGHVAAGSTLARRKRSAGAGSHCQKTSLRVNFEDIGWDSWIIAPKEYEAYECKGGCFFPLADDVTPTKHAIVQTLVHLKFPTKVGKACCVPTKLSPISVLYKDDMGVPTLKYHYEGMSVAECGCR

SEQ ID NO: 2 - protein, 426 aa, Artificial Sequence
  BMP-9 varient
MAWVWTLLFLMAAAQSIQAKPLQSWGRGSAGGNAHSPLGVPGGGLPEHTFNLKMFLENVKVDFLRSLNLSGVPSQDKTRVEPPQYMIDLYNRYTSDKSTTPASNIVRSFSMEDAISITATEDFPFQKHILLFNISIPRHEQITRAELRLYVSCQNHVDPSHDLKGSVVIYDVLDGTDAWDSATETKTFLVSQDIQDEGWETLEVSSAVKRWVRSDSTKSKNKLEVTVESHRKGCDTLDISVPPGSRNLPFFVVFSNDHSSGTKETRLELREMISHEQESVLKKLSKDGSTEAGESSHEEDTDGHVAAGSTLARRKRSAGAGSHCQKTSLRVNFEAIGWDSWIIAPKEYEAYECKGGCFFPLADDVTPTKHAIVQTLVHLKFPTKVGKACCVPTKLSPISVLYKDDMGVPTLKYHYEGMSVAECGCR

SEQ ID NO: 3 - protein, 426 aa, Artificial Sequence
  BMP-9 varient
MAWVWTLLFLMAAAQSIQAKPLQSWGRGSAGGNAHSPLGVPGGGLPEHTFNLKMFLENVKVDFLRSLNLSGVPSQDKTRVEPPQYMIDLYNRYTSDKSTTPASNIVRSFSMEDAISITATEDFPFQKHILLFNISIPRHEQITRAELRLYVSCQNHVDPSHDLKGSVVIYDVLDGTDAWDSATETKTFLVSQDIQDEGWETLEVSSAVKRWVRSDSTKSKNKLEVTVESHRKGCDTLDISVPPGSRNLPFFVVFSNDHSSGTKETRLELREMISHEQESVLKKLSKDGSTEAGESSHEEDTDGHVAAGSTLARRKRSAGAGSHCQKTSLRVNFEDIEWDSWIIAPKEYEAYECKGGCFFPLADDVTPTKHAIVQTLVHLKFPTKVGKACCVPTKLSPISVLYKDDMGVPTLKYHYEGMSVAECGCR

SEQ ID NO: 4 - protein, 426 aa, Artificial Sequence
  BMP-9 varient
MAWVWTLLFLMAAAQSIQAKPLQSWGRGSAGGNAHSPLGVPGGGLPEHTFNLKMFLENVKVDFLRSLNLSGVPSQDKTRVEPPQYMIDLYNRYTSDKSTTPASNIVRSFSMEDAISITATEDFPFQKHILLFNISIPRHEQITRAELRLYVSCQNHVDPSHDLKGSVVIYDVLDGTDAWDSATETKTFLVSQDIQDEGWETLEVSSAVKRWVRSDSTKSKNKLEVTVESHRKGCDTLDISVPPGSRNLPFFVVFSNDHSSGTKETRLELREMISHEQESVLKKLSKDGSTEAGESSHEEDTDGHVAAGSTLARRKRSAGAGSHCQKTSLRVNFEDIGWDSWIIAPKEYEAYECKGGCFFPLADEVTPTKHAIVQTLVHLKFPTKVGKACCVPTKLSPISVLYKDDMGVPTLKYHYEGMSVAECGCR

SEQ ID NO: 5 - protein, 426 aa, Artificial Sequence
  BMP-9 varient
MAWVWTLLFLMAAAQSIQAKPLQSWGRGSAGGNAHSPLGVPGGGLPEHTFNLKMFLENVKVDFLRSLNLSGVPSQDKTRVEPPQYMIDLYNRYTSDKSTTPASNIVRSFSMEDAISITATEDFPFQKHILLFNISIPRHEQITRAELRLYVSCQNHVDPSHDLKGSVVIYDVLDGTDAWDSATETKTFLVSQDIQDEGWETLEVSSAVKRWVRSDSTKSKNKLEVTVESHRKGCDTLDISVPPGSRNLPFFVVFSNDHSSGTKETRLELREMISHEQESVLKKLSKDGSTEAGESSHEEDTDGHVAAGSTLARRKRSAGAGSHCQKTSLRVNFEDIGWDSWIIAPKEYEAYECKGGCFFPLADDVTPTKHDIVQTLVHLKFPTKVGKACCVPTKLSPISVLYKDDMGVPTLKYHYEGMSVAECGCR

SEQ ID NO: 6 - protein, 426 aa, Artificial Sequence
  BMP-9 varient
MAWVWTLLFLMAAAQSIQAKPLQSWGRGSAGGNAHSPLGVPGGGLPEHTFNLKMFLENVKVDFLRSLNLSGVPSQDKTRVEPPQYMIDLYNRYTSDKSTTPASNIVRSFSMEDAISITATEDFPFQKHILLFNISIPRHEQITRAELRLYVSCQNHVDPSHDLKGSVVIYDVLDGTDAWDSATETKTFLVSQDIQDEGWETLEVSSAVKRWVRSDSTKSKNKLEVTVESHRKGCDTLDISVPPGSRNLPFFVVFSNDHSSGTKETRLELREMISHEQESVLKKLSKDGSTEAGESSHEEDTDGHVAAGSTLARRKRSAGAGSHCQKTSLRVNFEDIGWDSWIIAPKEYEAYECKGGCFFPLADDVTPTKHAIVQTLVHLKFPTKVGKACCVPTKLSPISVLYKDEMGVPTLKYHYEGMSVAECGCR

SEQ ID NO: 7 - protein, 426 aa, Artificial Sequence
  BMP-9 varient
MAWVWTLLFLMAAAQSIQAKPLQSWGRGSAGGNAHSPLGVPGGGLPEHTFNLKMFLENVKVDFLRSLNLSGVPSQDKTRVEPPQYMIDLYNRYTSDKSTTPASNIVRSFSMEDAISITATEDFPFQKHILLFNISIPRHEQITRAELRLYVSCQNHVDPSHDLKGSVVIYDVLDGTDAWDSATETKTFLVSQDIQDEGWETLEVSSAVKRWVRSDSTKSKNKLEVTVESHRKGCDTLDISVPPGSRNLPFFVVFSNDHSSGTKETRLELREMISHEQESVLKKLSKDGSTEAGESSHEEDTDGHVAAGSTLARRKRSAGAGSHCQKTSLRVNFEDIGWDSWIIAPKEYEAYECKGGCFFPLADDVTPTKHAIVQTLVHLKFPTKVGKACCVPTKLSPISVLYKDNMGVPTLKYHYEGMSVAECGCR

SEQ ID NO: 8 - protein, 426 aa, Artificial Sequence
  BMP-9 varient
MAWVWTLLFLMAAAQSIQAKPLQSWGRGSAGGNAHSPLGVPGGGLPEHTFNLKMFLENVKVDFLRSLNLSGVPSQDKTRVEPPQYMIDLYNRYTSDKSTTPASNIVRSFSMEDAISITATEDFPFQKHILLFNISIPRHEQITRAELRLYVSCQNHVDPSHDLKGSVVIYDVLDGTDAWDSATETKTFLVSQDIQDEGWETLEVSSAVKRWVRSDSTKSKNKLEVTVESHRKGCDTLDISVPPGSRNLPFFVVFSNDHSSGTKETRLELREMISHEQESVLKKLSKDGSTEAGESSHEEDTDGHVAAGSTLARRKRSAGAGSHCQKTSLRVNFEDIGWDSWIIAPKEYEAYECKGGCFFPLADDVTPTKHAIVQTLVHLKFPTKVGKACCVPTKLSPISVLYKDQMGVPTLKYHYEGMSVAECGCR

SEQ ID NO: 9 - protein, 426 aa, Artificial Sequence
  BMP-9 varient
MAWVWTLLFLMAAAQSIQAKPLQSWGRGSAGGNAHSPLGVPGGGLPEHTFNLKMFLENVKVDFLRSLNLSGVPSQDKTRVEPPQYMIDLYNRYTSDKSTTPASNIVRSFSMEDAISITATEDFPFQKHILLFNISIPRHEQITRAELRLYVSCQNHVDPSHDLKGSVVIYDVLDGTDAWDSATETKTFLVSQDIQDEGWETLEVSSAVKRWVRSDSTKSKNKLEVTVESHRKGCDTLDISVPPGSRNLPFFVVFSNDHSSGTKETRLELREMISHEQESVLKKLSKDGSTEAGESSHEEDTDGHVAAGSTLARRKRSAGAGSHCQKTSLRVNFEDIGWDSWIIAPKEYEAYECKGGCFFPLADDVTPTKHAIVQTLVHLKFPTKVGKACCVPTKLSPISVLYKDDMGVPTLKYHWEGMSVAECGCR

SEQ ID NO: 10 - protein, 426 aa, Artificial Sequence
  BMP-9 varient
MAWVWTLLFLMAAAQSIQAKPLQSWGRGSAGGNAHSPLGVPGGGLPEHTFNLKMFLENVKVDFLRSLNLSGVPSQDKTRVEPPQYMIDLYNRYTSDKSTTPASNIVRSFSMEDAISITATEDFPFQKHILLFNISIPRHEQITRAELRLYVSCQNHVDPSHDLKGSVVIYDVLDGTDAWDSATETKTFLVSQDIQDEGWETLEVSSAVKRWVRSDSTKSKNKLEVTVESHRKGCDTLDISVPPGSRNLPFFVVFSNDHSSGTKETRLELREMISHEQESVLKKLSKDGSTEAGESSHEEDTDGHVAAGSTLARRKRSAGAGSHCQKTSLRVNFEDIGWDSWIIAPKEYEAYECKGGCFFPKADDVTPTKHAIVQTLVHLKFPTKVGKACCVPTKLSPISVLYKDDMGVPTLKYHYEGMSVAECGCR

SEQ ID NO: 11 - protein, 426 aa, Artificial Sequence
  BMP-9 varient
MAWVWTLLFLMAAAQSIQAKPLQSWGRGSAGGNAHSPLGVPGGGLPEHTFNLKMFLENVKVDFLRSLNLSGVPSQDKTRVEPPQYMIDLYNRYTSDKSTTPASNIVRSFSMEDAISITATEDFPFQKHILLFNISIPRHEQITRAELRLYVSCQNHVDPSHDLKGSVVIYDVLDGTDAWDSATETKTFLVSQDIQDEGWETLEVSSAVKRWVRSDSTKSKNKLEVTVESHRKGCDTLDISVPPGSRNLPFFVVFSNDHSSGTKETRLELREMISHEQESVLKKLSKDGSTEAGESSHEEDTDGHVAAGSTLARRKRSAGAGSHCQKTSLRVNFEDIGWDSWIIAPKEYEAYECKGGCFFPLANDVTPTKHAIVQTLVHLKFPTKVGKACCVPTKLSPISVLYKDDMGVPTLKYHYEGMSVAECGCR

SEQ ID NO: 12 - protein, 426 aa, Artificial Sequence
  BMP-9 varient
MAWVWTLLFLMAAAQSIQAKPLQSWGRGSAGGNAHSPLGVPGGGLPEHTFNLKMFLENVKVDFLRSLNLSGVPSQDKTRVEPPQYMIDLYNRYTSDKSTTPASNIVRSFSMEDAISITATEDFPFQKHILLFNISIPRHEQITRAELRLYVSCQNHVDPSHDLKGSVVIYDVLDGTDAWDSATETKTFLVSQDIQDEGWETLEVSSAVKRWVRSDSTKSKNKLEVTVESHRKGCDTLDISVPPGSRNLPFFVVFSNDHSSGTKETRLELREMISHEQESVLKKLSKDGSTEAGESSHEEDTDGHVAAGSTLARRKRSAGAGSHCQKTSLRVNFEDIGWDSWIIAPKEYEAYECKGGCFFPLAQDVTPTKHAIVQTLVHLKFPTKVGKACCVPTKLSPISVLYKDDMGVPTLKYHYEGMSVAECGCR

SEQ ID NO: 13 - protein, 426 aa, Artificial Sequence
  BMP-9 varient
MAWVWTLLFLMAAAQSIQAKPLQSWGRGSAGGNAHSPLGVPGGGLPEHTFNLKMFLENVKVDFLRSLNLSGVPSQDKTRVEPPQYMIDLYNRYTSDKSTTPASNIVRSFSMEDAISITATEDFPFQKHILLFNISIPRHEQITRAELRLYVSCQNHVDPSHDLKGSVVIYDVLDGTDAWDSATETKTFLVSQDIQDEGWETLEVSSAVKRWVRSDSTKSKNKLEVTVESHRKGCDTLDISVPPGSRNLPFFVVFSNDHSSGTKETRLELREMISHEQESVLKKLSKDGSTEAGESSHEEDTDGHVAAGSTLARRKRSAGAGSHCQKTSLRVNFEDIGWDSWIIAPKEYEAYECKGGCFFPLADDVTPTKHPIVQTLVHLKFPTKVGKACCVPTKLSPISVLYKDDMGVPTLKYHYEGMSVAECGCR

SEQ ID NO: 14 - protein, 426 aa, Artificial Sequence
  BMP-9 varient
MAWVWTLLFLMAAAQSIQAKPLQSWGRGSAGGNAHSPLGVPGGGLPEHTFNLKMFLENVKVDFLRSLNLSGVPSQDKTRVEPPQYMIDLYNRYTSDKSTTPASNIVRSFSMEDAISITATEDFPFQKHILLFNISIPRHEQITRAELRLYVSCQNHVDPSHDLKGSVVIYDVLDGTDAWDSATETKTFLVSQDIQDEGWETLEVSSAVKRWVRSDSTKSKNKLEVTVESHRKGCDTLDISVPPGSRNLPFFVVFSNDHSSGTKETRLELREMISHEQESVLKKLSKDGSTEAGESSHEEDTDGHVAAGSTLARRKRSAGAGSHCQKTSLRVNFEDIGWDSWIIAPKEYEAYECKGGCFFPLADDVTPTKHARVQTLVHLKFPTKVGKACCVPTKLSPISVLYKDDMGVPTLKYHYEGMSVAECGCR

SEQ ID NO: 15 - protein, 426 aa, Artificial Sequence
  BMP-9 varient
MAWVWTLLFLMAAAQSIQAKPLQSWGRGSAGGNAHSPLGVPGGGLPEHTFNLKMFLENVKVDFLRSLNLSGVPSQDKTRVEPPQYMIDLYNRYTSDKSTTPASNIVRSFSMEDAISITATEDFPFQKHILLFNISIPRHEQITRAELRLYVSCQNHVDPSHDLKGSVVIYDVLDGTDAWDSATETKTFLVSQDIQDEGWETLEVSSAVKRWVRSDSTKSKNKLEVTVESHRKGCDTLDISVPPGSRNLPFFVVFSNDHSSGTKETRLELREMISHEQESVLKKLSKDGSTEAGESSHEEDTDGHVAAGSTLARRKRSAGAGSHCQKTSLRVNFEDIGWDSWIIAPKEYEAYECKGGCFFPLADDVTPTKHAIVQTRVHLKFPTKVGKACCVPTKLSPISVLYKDDMGVPTLKYHYEGMSVAECGCR

SEQ ID NO: 16 - protein, 426 aa, Artificial Sequence
  BMP-9 varient
MAWVWTLLFLMAAAQSIQAKPLQSWGRGSAGGNAHSPLGVPGGGLPEHTFNLKMFLENVKVDFLRSLNLSGVPSQDKTRVEPPQYMIDLYNRYTSDKSTTPASNIVRSFSMEDAISITATEDFPFQKHILLFNISIPRHEQITRAELRLYVSCQNHVDPSHDLKGSVVIYDVLDGTDAWDSATETKTFLVSQDIQDEGWETLEVSSAVKRWVRSDSTKSKNKLEVTVESHRKGCDTLDISVPPGSRNLPFFVVFSNDHSSGTKETRLELREMISHEQESVLKKLSKDGSTEAGESSHEEDTDGHVAAGSTLARRKRSAGAGSHCQKTSLRVNFEDIGWDSWIIAPKEYEAYECKGGCFFPLADDVTPTKHHKVQTLVHLKFPTKVGKACCVPTKLSPISVLYKDDMGVPTLKYHYEGMSVAECGCR

SEQ ID NO: 17 - protein, 426 aa, Artificial Sequence
  BMP-9 varient
MAWVWTLLFLMAAAQSIQAKPLQSWGRGSAGGNAHSPLGVPGGGLPEHTFNLKMFLENVKVDFLRSLNLSGVPSQDKTRVEPPQYMIDLYNRYTSDKSTTPASNIVRSFSMEDAISITATEDFPFQKHILLFNISIPRHEQITRAELRLYVSCQNHVDPSHDLKGSVVIYDVLDGTDAWDSATETKTFLVSQDIQDEGWETLEVSSAVKRWVRSDSTKSKNKLEVTVESHRKGCDTLDISVPPGSRNLPFFVVFSNDHSSGTKETRLELREMISHEQESVLKKLSKDGSTEAGESSHEEDTDGHVAAGSTLARRKRSAGAGSHCQKTSLRVNFEDIGWDSWIIAPKEYEAYECKGGCFFPLADDVTPTKRRKVQTLVHLKFPTKVGKACCVPTKLSPISVLYKDDMGVPTLKYHYEGMSVAECGCR

SEQ ID NO: 18 - protein, 426 aa, Artificial Sequence
  BMP-9 varient
MAWVWTLLFLMAAAQSIQAKPLQSWGRGSAGGNAHSPLGVPGGGLPEHTFNLKMFLENVKVDFLRSLNLSGVPSQDKTRVEPPQYMIDLYNRYTSDKSTTPASNIVRSFSMEDAISITATEDFPFQKHILLFNISIPRHEQITRAELRLYVSCQNHVDPSHDLKGSVVIYDVLDGTDAWDSATETKTFLVSQDIQDEGWETLEVSSAVKRWVRSDSTKSKNKLEVTVESHRKGCDTLDISVPPGSRNLPFFVVFSNDHSSGTKETRLELREMISHEQESVLKKLSKDGSTEAGESSHEEDTDGHVAAGSTLARRKRSAGAGSHCQKTSLRVNFEDIGWDSWIIAPKEYEAYECKGGCFFPLADDVTPTKHRKVRTRVHLKFPTKVGKACCVPTKLSPISVLYKDDMGVPTLKYHYEGMSVAECGCR

SEQ ID NO: 19 - protein, 426 aa, Artificial Sequence
  BMP-9 varient
MAWVWTLLFLMAAAQSIQAKPLQSWGRGSAGGNAHSPLGVPGGGLPEHTFNLKMFLENVKVDFLRSLNLSGVPSQDKTRVEPPQYMIDLYNRYTSDKSTTPASNIVRSFSMEDAISITATEDFPFQKHILLFNISIPRHEQITRAELRLYVSCQNHVDPSHDLKGSVVIYDVLDGTDAWDSATETKTFLVSQDIQDEGWETLEVSSAVKRWVRSDSTKSKNKLEVTVESHRKGCDTLDISVPPGSRNLPFFVVFSNDHSSGTKETRLELREMISHEQESVLKKLSKDGSTEAGESSHEEDTDGHVAAGSTLARRKRSAGAGSHCQKTSLRVNFEDIGWDSWIIAPKEYEAYECKGGCFFPLADDVTPTKPRIVQTLVHLKFPTKVGKACCVPTKLSPISVLYKDDMGVPTLKYHYEGMSVAECGCR

SEQ ID NO: 20 - protein, 426 aa, Artificial Sequence
  BMP-9 varient
MAWVWTLLFLMAAAQSIQAKPLQSWGRGSAGGNAHSPLGVPGGGLPEHTFNLKMFLENVKVDFLRSLNLSGVPSQDKTRVEPPQYMIDLYNRYTSDKSTTPASNIVRSFSMEDAISITATEDFPFQKHILLFNISIPRHEQITRAELRLYVSCQNHVDPSHDLKGSVVIYDVLDGTDAWDSATETKTFLVSQDIQDEGWETLEVSSAVKRWVRSDSTKSKNKLEVTVESHRKGCDTLDISVPPGSRNLPFFVVFSNDHSSGTKETRLELREMISHEQESVLKKLSKDGSTEAGESSHEEDTDGHVAAGSTLARRKRSAGAGSHCQKTSLRVNFEDIGWDSWIIAPKEYEAYECKGGCFWPLADDVTPTKHAIVQTLVHLKYPTKVGKACCVPTKLSPISVLYKDDMGVPTLKYHYEGMSVAECGCR

SEQ ID NO: 21 - protein, 426 aa, Artificial Sequence
  BMP-9 varient
MAWVWTLLFLMAAAQSIQAKPLQSWGRGSAGGNAHSPLGVPGGGLPEHTFNLKMFLENVKVDFLRSLNLSGVPSQDKTRVEPPQYMIDLYNRYTSDKSTTPASNIVRSFSMEDAISITATEDFPFQKHILLFNISIPRHEQITRAELRLYVSCQNHVDPSHDLKGSVVIYDVLDGTDAWDSATETKTFLVSQDIQDEGWETLEVSSAVKRWVRSDSTKSKNKLEVTVESHRKGCDTLDISVPPGSRNLPFFVVFSNDHSSGTKETRLELREMISHEQESVLKKLSKDGSTEAGESSHEEDTDGHVAAGSTLARRKRSAGAGSHCQKTSLRVNFEDIGWDSWIIAPKEYEAYECKGGCFFPCADDVTPTKHCIDQTLDHLKFPTKVGKACCVPTKLSPISVLYKDDMGVPTLKYHYEGMSVAECGCR

SEQ ID NO: 22 - protein, 426 aa, Artificial Sequence
  BMP-9 varient
MAWVWTLLFLMAAAQSIQAKPLQSWGRGSAGGNAHSPLGVPGGGLPEHTFNLKMFLENVKVDFLRSLNLSGVPSQDKTRVEPPQYMIDLYNRYTSDKSTTPASNIVRSFSMEDAISITATEDFPFQKHILLFNISIPRHEQITRAELRLYVSCQNHVDPSHDLKGSVVIYDVLDGTDAWDSATETKTFLVSQDIQDEGWETLEVSSAVKRWVRSDSTKSKNKLEVTVESHRKGCDTLDISVPPGSRNLPFFVVFSNDHSSGTKETRLELREMISHEQESVLKKLSKDGSTEAGESSHEEDTDGHVAAGSTLARRKRSAGAGSHCQKTSLRVNFEDIGWDSWIIAPKEYEAYECKGGCFFPLADDVTPTKHAIVQTLVHLKCGGKVGKACCVPTKLSPISVLYKDDMGVPTLKYHYEGMSVAECGCR

SEQ ID NO: 23 - protein, 426 aa, Artificial Sequence
  BMP-9 varient
MAWVWTLLFLMAAAQSIQAKPLQSWGRGSAGGNAHSPLGVPGGGLPEHTFNLKMFLENVKVDFLRSLNLSGVPSQDKTRVEPPQYMIDLYNRYTSDKSTTPASNIVRSFSMEDAISITATEDFPFQKHILLFNISIPRHEQITRAELRLYVSCQNHVDPSHDLKGSVVIYDVLDGTDAWDSATETKTFLVSQDIQDEGWETLEVSSAVKRWVRSDSTKSKNKLEVTVESHRKGCDTLDISVPPGSRNLPFFVVFSNDHSSGTKETRLELREMISHEQESVLKKLSKDGSTEAGESSHEEDTDGHVAAGSTLARRKRSAGAGSHCQKTSLRVNFEDIGWDSWIIAPKEYEAYECKGGCFFPCADDVTPTKHCIDQTLDHLKFPTKVGKDCCVPTKISPISVLWKDDMGVPTLKYHYEGMSVAECGCR

SEQ ID NO: 24 - protein, 426 aa, Artificial Sequence
  BMP-9 varient
MAWVWTLLFLMAAAQSIQAKPLQSWGRGSAGGNAHSPLGVPGGGLPEHTFNLKMFLENVKVDFLRSLNLSGVPSQDKTRVEPPQYMIDLYNRYTSDKSTTPASNIVRSFSMEDAISITATEDFPFQKHILLFNISIPRHEQITRAELRLYVSCQNHVDPSHDLKGSVVIYDVLDGTDAWDSATETKTFLVSQDIQDEGWETLEVSSAVKRWVRSDSTKSKNKLEVTVESHRKGCDTLDISVPPGSRNLPFFVVFSNDHSSGTKETRLELREMISHEQESVLKKLSKDGSTEAGESSHEEDTDGHVAAGSTLARRKRSAGAGSHCQKTSLRVNFEDIGWDSWIIAPKEYEAYECKGGCFFPLADDVTPTKHAIVQTLVHLKCGGKVGKACCAPTPLSPISVLWKDDMGVPTLKYHYEGMSVAECGCR

SEQ ID NO: 25 - protein, 426 aa, Artificial Sequence
  BMP-9 varient
MAWVWTLLFLMAAAQSIQAKPLQSWGRGSAGGNAHSPLGVPGGGLPEHTFNLKMFLENVKVDFLRSLNLSGVPSQDKTRVEPPQYMIDLYNRYTSDKSTTPASNIVRSFSMEDAISITATEDFPFQKHILLFNISIPRHEQITRAELRLYVSCQNHVDPSHDLKGSVVIYDVLDGTDAWDSATETKTFLVSQDIQDEGWETLEVSSAVKRWVRSDSTKSKNKLEVTVESHRKGCDTLDISVPPGSRNLPFFVVFSNDHSSGTKETRLELREMISHEQESVLKKLSKDGSTEAGESSHEEDTDGHVAAGSTLARRKRSAGAGSHCQKTSLRVNFEDIGWDSWIIAPKEYEAYECKGGCFFPLAADVTPTKHAIVQTLVHLKFPTKVGKACCVPTKLSPISVLYKDDMGVPTLKYHYEGMSVAECGCR

SEQ ID NO: 26 - protein, 426 aa, Artificial Sequence
  BMP-9 varient
MAWVWTLLFLMAAAQSIQAKPLQSWGRGSAGGNAHSPLGVPGGGLPEHTFNLKMFLENVKVDFLRSLNLSGVPSQDKTRVEPPQYMIDLYNRYTSDKSTTPASNIVRSFSMEDAISITATEDFPFQKHILLFNISIPRHEQITRAELRLYVSCQNHVDPSHDLKGSVVIYDVLDGTDAWDSATETKTFLVSQDIQDEGWETLEVSSAVKRWVRSDSTKSKNKLEVTVESHRKGCDTLDISVPPGSRNLPFFVVFSNDHSSGTKETRLELREMISHEQESVLKKLSKDGSTEAGESSHEEDTDGHVAAGSTLARRKRSAGAGSHCQKTSLRVNFEDIGWDSWIIAPKEYEAYECKGGCFFPLADDVTPTKHAIVQTLVHLKFPTKVGKACCVPTKLSPISVLYKDAMGVPTLKYHYEGMSVAECGCR

SEQ ID NO: 27 - protein, 426 aa, Artificial Sequence
  BMP-9 varient
MAWVWTLLFLMAAAQSIQAKPLQSWGRGSAGGNAHSPLGVPGGGLPEHTFNLKMFLENVKVDFLRSLNLSGVPSQDKTRVEPPQYMIDLYNRYTSDKSTTPASNIVRSFSMEDAISITATEDFPFQKHILLFNISIPRHEQITRAELRLYVSCQNHVDPSHDLKGSVVIYDVLDGTDAWDSATETKTFLVSQDIQDEGWETLEVSSAVKRWVRSDSTKSKNKLEVTVESHRKGCDTLDISVPPGSRNLPFFVVFSNDHSSGTKETRLELREMISHEQESVLKKLSKDGSTEAGESSHEEDTDGHVAAGSTLARRKRSAGAGSHCQKTSLRVNFEDIGWDSWIIAPKEYEAYECKGGCFFPLAEDVTPTKHAIVQTLVHLKFPTKVGKACCVPTKLSPISVLYKDDMGVPTLKYHYEGMSVAECGCR

SEQ ID NO: 28 - protein, 426 aa, Artificial Sequence
  BMP-9 varient
MAWVWTLLFLMAAAQSIQAKPLQSWGRGSAGGNAHSPLGVPGGGLPEHTFNLKMFLENVKVDFLRSLNLSGVPSQDKTRVEPPQYMIDLYNRYTSDKSTTPASNIVRSFSMEDAISITATEDFPFQKHILLFNISIPRHEQITRAELRLYVSCQNHVDPSHDLKGSVVIYDVLDGTDAWDSATETKTFLVSQDIQDEGWETLEVSSAVKRWVRSDSTKSKNKLEVTVESHRKGCDTLDISVPPGSRNLPFFVVFSNDHSSGTKETRLELREMISHEQESVLKKLSKDGSTEAGESSHEEDTDGHVAAGSTLARRKRSAGAGSHCQKTSLRVNFEDIGWDSWIIAPKEYEAYECKGGCFFPLAADVTPTKHAIVQTLVHLKFPTKVGKACCVPTKLSPISVLYKDAMGVPTLKYHYEGMSVAECGCR

SEQ ID NO: 29 - protein, 24 aa, Artificial Sequence
  BMP-9 varient
FFPLADDVTPTKHAIVQTLVHLKF

SEQ ID NO: 30 - protein, 243 aa, Artificial Sequence
  Fc
MAWVWTLLFLMAAAQSIQAHTCPPCPAPELLGGPSVFLFPPKPKDTLMISRTPEVTCVVVDVSHEDPEVKFNWYVDGVEVHNAKTKPREEQYNSTYRVVSVLTVLHQDWLNGKEYKCKVSNKALPAPIEKTISKAKGQPREPQVYTLPPSRDELTKNQVSLTCLVKGFYPSDIAVEWESNGQPENNYKTTPPVLDSDGSFFLYSKLTVDKSRWQQGNVFSCSVMHEALHNHYTQKSLSLSPGK

SEQ ID NO: 31 - protein, 15 aa, Artificial Sequence
  Linker
GGGGSGGGGSGGGGS

SEQ ID NO: 32 - protein, 368 aa, Artificial Sequence
  BMP-Fc fusion
MAWVWTLLFLMAAAQSIQAHTCPPCPAPELLGGPSVFLFPPKPKDTLMISRTPEVTCVVVDVSHEDPEVKFNWYVDGVEVHNAKTKPREEQYNSTYRVVSVLTVLHQDWLNGKEYKCKVSNKALPAPIEKTISKAKGQPREPQVYTLPPSRDELTKNQVSLTCLVKGFYPSDIAVEWESNGQPENNYKTTPPVLDSDGSFFLYSKLTVDKSRWQQGNVFSCSVMHEALHNHYTQKSLSLSPGKGGGGSGGGGSGGGGSSAGAGSHCQKTSLRVNFEDIGWDSWIIAPKEYEAYECKGGCFFPLADDVTPTKHAIVQTLVHLKFPTKVGKACCVPTKLSPISVLYKDDMGVPTLKYHYEGMSVAECGCR

SEQ ID NO: 33 - protein, 665 aa, Artificial Sequence
  BMP-Fc fusion
MAWVWTLLFLMAAAQSIQAKPLQSWGRGSAGGNAHSPLGVPGGGLPEHTFNLKMFLENVKVDFLRSLNLSGVPSQDKTRVEPPQYMIDLYNRYTSDKSTTPASNIVRSFSMEDAISITATEDFPFQKHILLFNISIPRHEQITRAELRLYVSCQNHVDPSHDLKGSVVIYDVLDGTDAWDSATETKTFLVSQDIQDEGWETLEVSSAVKRWVRSDSTKSKNKLEVTVESHRKGCDTLDISVPPGSRNLPFFVVFSNDHSSGTKETRLELREMISHEQESVLKKLSKDGSTEAGESSHEEDTDGHVAAGSTLARRKRSAGAGSHCQKTSLRVNFEDIGWDSWIIAPKEYEAYECKGGCFFPLADDVTPTKHAIVQTLVHLKFPTKVGKACCVPTKLSPISVLYKDDMGVPTLKYHYEGMSVAECGCRGGGGSGGGGSGGGGSHTCPPCPAPELLGGPSVFLFPPKPKDTLMISRTPEVTCVVVDVSHEDPEVKFNWYVDGVEVHNAKTKPREEQYNSTYRVVSVLTVLHQDWLNGKEYKCKVSNKALPAPIEKTISKAKGQPREPQVYTLPPSRDELTKNQVSLTCLVKGFYPSDIAVEWESNGQPENNYKTTPPVLDSDGSFFLYSKLTVDKSRWQQGNVFSCSVMHEALHNHYTQKSLSLSPGK